European Patent Application EP 4 219 687 A1, published August 2, 2023. Title: METHODS FOR ISOLATING, CULTURING, AND GENETICALLY ENGINEERING IMMUNE CELL POPULATIONS FOR ADOPTIVE THERAPY. Applicant: Juno Therapeutics, Inc. Application US. The sequence listing filed with the application follows.

SEQUENCE LISTING (19 sequences)

SEQ ID NO: 1 - skipped

SEQ ID NO: 2 - protein, 4 aa, synthetic construct
  REGION 1..4: note = Synthetic
  REGION 1..4: note = Streptavidin-binding peptide
HPQF

SEQ ID NO: 3 - protein, 8 aa, synthetic construct
  REGION 1..8: note = Synthetic
  REGION 1..8: note = Streptavidin-binding peptide
  VARIANT 1: note = Xaa = Trp, Lys or Arg
  VARIANT 2: note = Xaa = any amino acid
  VARIANT 7: note = Xaa = Gly or Glu
  VARIANT 8: note = Xaa = Gly, Lys or Arg
XXHPQFXX

SEQ ID NO: 4 - protein, 8 aa, synthetic construct
  REGION 1..8: note = Synthetic
  REGION 1..8: note = Streptavidin-binding peptide
  VARIANT 2: note = Xaa = any amino acid
  VARIANT 7: note = Xaa = Gly or Glu
  VARIANT 8: note = Xaa = Gly, Lys or Arg
WXHPQFXX

SEQ ID NO: 5 - protein, 8 aa, synthetic construct
  REGION 1..8: note = Synthetic
  REGION 1..8: note = Streptavidin-binding peptide
WRHPQFGG

SEQ ID NO: 6 - protein, 8 aa, synthetic construct
  REGION 1..8: note = Synthetic
  REGION 1..8: note = Strep-tag (registered trademark) II
WSHPQFEK

SEQ ID NO: 7 - protein, 28 aa, synthetic construct
  REGION 1..28: note = Synthetic
  REGION 1..28: note = Sequential modules of streptavidin-binding peptide
  VARIANT 9..20: note = Xaa at positions 9-20 may be any amino acid and 4 of them may be absent
WSHPQFEKXXXXXXXXXXXXWSHPQFEK

SEQ ID NO: 8 - protein, 28 aa, synthetic construct
  REGION 1..28: note = Synthetic
  REGION 1..28: note = Sequential modules of streptavidin-binding peptide
  VARIANT 9..12: note = These amino acids may be absent
WSHPQFEKGGGSGGGSGGGSWSHPQFEK

SEQ ID NO: 9 - protein, 30 aa, synthetic construct
  REGION 1..30: note = Synthetic
  REGION 1..30: note = Twin-Strep-Tag
SAWSHPQFEKGGGSGGGSGGGSWSHPQFEK

SEQ ID NO: 10 - protein, 30 aa, synthetic construct
  REGION 1..30: note = Synthetic
  REGION 1..30: note = Twin-Strep-Tag
SAWSHPQFEKGGGSGGGSGGSAWSHPQFEK

SEQ ID NO: 11 - protein, 159 aa, Streptomyces Avidinii
  REGION 1..159: note = Streptavidin
DPSKDSKAQVSAAEAGITGTWYNQLGSTFIVTAGADGALTGTYESAVGNAESRYVLTGRYDSAPATDGSGTALGWTVAWKNNYRNAHSATTWSGQYVGGAEARINTQWLLTSGTTEANAWKSTLVGHDTFTKVKPSAASIDAAKKAGVNNGNPLDAVQQ

SEQ ID NO: 12 - protein, 159 aa, Streptomyces Avidinii
  REGION 1..159: note = Mutein Streptavidin Val44-Thr45-Ala46-Arg47
DPSKDSKAQVSAAEAGITGTWYNQLGSTFIVTAGADGALTGTYVTARGNAESRYVLTGRYDSAPATDGSGTALGWTVAWKNNYRNAHSATTWSGQYVGGAEARINTQWLLTSGTTEANAWKSTLVGHDTFTKVKPSAASIDAAKKAGVNNGNPLDAVQQ

SEQ ID NO: 13 - protein, 159 aa, Streptomyces Avidinii
  REGION 1..159: note = Mutein Streptavidin Ile44-Gly45-Ala-46-Arg47
DPSKDSKAQVSAAEAGITGTWYNQLGSTFIVTAGADGALTGTYIGARGNAESRYVLTGRYDSAPATDGSGTALGWTVAWKNNYRNAHSATTWSGQYVGGAEARINTQWLLTSGTTEANAWKSTLVGHDTFTKVKPSAASIDAAKKAGVNNGNPLDAVQQ

SEQ ID NO: 14 - protein, 126 aa, Streptomyces Avidinii
  REGION 1..126: note = Minimal streptavidin
EAGITGTWYNQLGSTFIVTAGADGALTGTYESAVGNAESRYVLTGRYDSAPATDGSGTALGWTVAWKNNYRNAHSATTWSGQYVGGAEARINTQWLLTSGTTEANAWKSTLVGHDTFTKVKPSAAS

SEQ ID NO: 15 - protein, 126 aa, Streptomyces Avidinii
  REGION 1..126: note = Mutein Streptavidin Val44-Thr45-Ala46-Arg47
EAGITGTWYNQLGSTFIVTAGADGALTGTYVTARGNAESRYVLTGRYDSAPATDGSGTALGWTVAWKNNYRNAHSATTWSGQYVGGAEARINTQWLLTSGTTEANAWKSTLVGHDTFTKVKPSAAS

SEQ ID NO: 16 - protein, 126 aa, Streptomyces Avidinii
  REGION 1..126: note = Mutein Streptavidin Ile44-Gly45-Ala-46-Arg47
EAGITGTWYNQLGSTFIVTAGADGALTGTYIGARGNAESRYVLTGRYDSAPATDGSGTALGWTVAWKNNYRNAHSATTWSGQYVGGAEARINTQWLLTSGTTEANAWKSTLVGHDTFTKVKPSAAS

SEQ ID NO: 17 - protein, 28 aa, synthetic construct
  REGION 1..28: note = Synthetic
  REGION 1..28: note = Twin Strep-tag
WSHPQFEKGGGSGGGSGGGSWSHPQFEK

SEQ ID NO: 18 - protein, 24 aa, synthetic construct
  REGION 1..24: note = Synthetic
  REGION 1..24: note = Twin Strep-tag
WSHPQFEKGGGSGGGSWSHPQFEK

SEQ ID NO: 19 - protein, 28 aa, synthetic construct
  REGION 1..28: note = Synthetic
  REGION 1..28: note = Twin Strep-tag
WSHPQFEKGGGSGGGSGGSAWSHPQFEK